European Patent Application EP 4 285 936 A1, published December 6, 2023. Title: ANTIBODY-DRUG CONJUGATE AND MEDICAL USE THEREOF. Applicant: SHANGHAI HANSOH BIOMEDICAL CO., LTD. JIANGSU HANSOH PHARMACEUTICAL GROUP CO., LTD. Application PCT/CN2022/073943. The sequence listing filed with the application follows.

SEQUENCE LISTING (23 sequences)

SEQ ID NO: 1 - protein, 121 aa, Artificial Sequence
  DOMAIN (1)..(121): mAb M1 VH
QVQLQQSGAELVRPGASVKLSCKALGYSFSDYEMHWVRQTPVHGLEWIGGIHPGSGGSAYNQKFKGKATLTVDKSSSTAYMELSSLTSEDSAVYYCTRLDYGYSWAWFPYWGQGTLVTVSA

SEQ ID NO: 2 - protein, 106 aa, Artificial Sequence
  DOMAIN (1)..(106): mAb M1 VL
EILLTQSPAIIVTSPGEKVTITCSASSSVIYMNWYQQKPGSSPKIWIYGISNLASGVPARFSGSGSGTSFSFTINSMEAEDVATYYCQQRSSYPLTFGAGTKLELK

SEQ ID NO: 3 - protein, 10 aa, Artificial Sequence
  DOMAIN (1)..(10): HCDR1
GYSFSDYEMH

SEQ ID NO: 4 - protein, 17 aa, Artificial Sequence
  DOMAIN (1)..(17): HCDR2
GIHPGSGGSAYNQKFKG

SEQ ID NO: 5 - protein, 14 aa, Artificial Sequence
  DOMAIN (1)..(14): HCDR3
TRLDYGYSWAWFPY

SEQ ID NO: 6 - protein, 10 aa, Artificial Sequence
  DOMAIN (1)..(10): LCDR1
SASSSVIYMN

SEQ ID NO: 7 - protein, 7 aa, Artificial Sequence
  DOMAIN (1)..(7): LCDR2
GISNLAS

SEQ ID NO: 8 - protein, 9 aa, Artificial Sequence
  DOMAIN (1)..(9): LCDR3
QQRSSYPLT

SEQ ID NO: 9 - protein, 121 aa, Artificial Sequence
  DOMAIN (1)..(121): humanized Ab VH1
QVQLVQSGAEVKKPGASVKVSCKASGYSFSDYEMHWVRQAPGQGLEWMGGIHPGSGGSAYNQKFKGRVTMTRDTSTSTVYMELSSLRSEDTAVYYCTRLDYGYSWAWFPYWGQGTLVTVSA

SEQ ID NO: 10 - protein, 121 aa, Artificial Sequence
  DOMAIN (1)..(121): humanized Ab VH2
QVQLVQSGAEVKKPGASVKVSCKASGYSFSDYEMHWVRQAPGQGLEWIGGIHPGSGGSAYNQKFKGRVTLTVDKSTSTAYMELSSLRSEDTAVYYCTRLDYGYSWAWFPYWGQGTLVTVSA

SEQ ID NO: 11 - protein, 121 aa, Artificial Sequence
  DOMAIN (1)..(121): humanized Ab VH3
QVQLVQSGAEVKKPGASVKVSCKASGYSFSDYEMHWVRQAPGQGLEWIGGIHPGSGGSAYNQKFKGKATLTVDKSTSTAYMELSSLRSEDTAVYYCTRLDYGYSWAWFPYWGQGTLVTVSA

SEQ ID NO: 12 - protein, 106 aa, Artificial Sequence
  DOMAIN (1)..(106): humanized Ab VL1
EIVLTQSPATLSLSPGERATLSCSASSSVIYMNWYQQKPGQAPRLLIYGISNLASGIPARFSGSGSGTDFTLTISSLEPEDFAVYYCQQRSSYPLTFGGGTKVEIK

SEQ ID NO: 13 - protein, 106 aa, Artificial Sequence
  DOMAIN (1)..(106): humanized Ab VL2
EIVLTQSPATLSLSPGERATLSCSASSSVIYMNWYQQKPGQSPKIWIYGISNLASGVPARFSGSGSGTDFTLTISSLEPEDFAVYYCQQRSSYPLTFGGGTKVEIK

SEQ ID NO: 14 - protein, 106 aa, Artificial Sequence
  DOMAIN (1)..(106): humanized Ab VL3
EILLTQSPATLSLSPGERATLTCSASSSVIYMNWYQQKPGSSPKIWIYGISNLASGVPARFSGSGSGTSFTLTISSLEPEDFAVYYCQQRSSYPLTFGGGTKVEIK

SEQ ID NO: 15 - protein, 451 aa, Artificial Sequence
  CHAIN (1)..(451): humanized Ab HC1
QVQLVQSGAEVKKPGASVKVSCKASGYSFSDYEMHWVRQAPGQGLEWMGGIHPGSGGSAYNQKFKGRVTMTRDTSTSTVYMELSSLRSEDTAVYYCTRLDYGYSWAWFPYWGQGTLVTVSAASTKGPSVFPLAPSSKSTSGGTAALGCLVKDYFPEPVTVSWNSGALTSGVHTFPAVLQSSGLYSLSSVVTVPSSSLGTQTYICNVNHKPSNTKVDKKVEPKSCDKTHTCPPCPAPELLGGPSVFLFPPKPKDTLMISRTPEVTCVVVDVSHEDPEVKFNWYVDGVEVHNAKTKPREEQYNSTYRVVSVLTVLHQDWLNGKEYKCKVSNKALPAPIEKTISKAKGQPREPQVYTLPPSRDELTKNQVSLTCLVKGFYPSDIAVEWESNGQPENNYKTTPPVLDSDGSFFLYSKLTVDKSRWQQGNVFSCSVMHEALHNHYTQKSLSLSPGK

SEQ ID NO: 16 - protein, 451 aa, Artificial Sequence
  CHAIN (1)..(451): humanized Ab HC2
QVQLVQSGAEVKKPGASVKVSCKASGYSFSDYEMHWVRQAPGQGLEWIGGIHPGSGGSAYNQKFKGRVTLTVDKSTSTAYMELSSLRSEDTAVYYCTRLDYGYSWAWFPYWGQGTLVTVSAASTKGPSVFPLAPSSKSTSGGTAALGCLVKDYFPEPVTVSWNSGALTSGVHTFPAVLQSSGLYSLSSVVTVPSSSLGTQTYICNVNHKPSNTKVDKKVEPKSCDKTHTCPPCPAPELLGGPSVFLFPPKPKDTLMISRTPEVTCVVVDVSHEDPEVKFNWYVDGVEVHNAKTKPREEQYNSTYRVVSVLTVLHQDWLNGKEYKCKVSNKALPAPIEKTISKAKGQPREPQVYTLPPSRDELTKNQVSLTCLVKGFYPSDIAVEWESNGQPENNYKTTPPVLDSDGSFFLYSKLTVDKSRWQQGNVFSCSVMHEALHNHYTQKSLSLSPGK

SEQ ID NO: 17 - protein, 451 aa, Artificial Sequence
  CHAIN (1)..(451): humanized Ab HC3
QVQLVQSGAEVKKPGASVKVSCKASGYSFSDYEMHWVRQAPGQGLEWIGGIHPGSGGSAYNQKFKGKATLTVDKSTSTAYMELSSLRSEDTAVYYCTRLDYGYSWAWFPYWGQGTLVTVSAASTKGPSVFPLAPSSKSTSGGTAALGCLVKDYFPEPVTVSWNSGALTSGVHTFPAVLQSSGLYSLSSVVTVPSSSLGTQTYICNVNHKPSNTKVDKKVEPKSCDKTHTCPPCPAPELLGGPSVFLFPPKPKDTLMISRTPEVTCVVVDVSHEDPEVKFNWYVDGVEVHNAKTKPREEQYNSTYRVVSVLTVLHQDWLNGKEYKCKVSNKALPAPIEKTISKAKGQPREPQVYTLPPSRDELTKNQVSLTCLVKGFYPSDIAVEWESNGQPENNYKTTPPVLDSDGSFFLYSKLTVDKSRWQQGNVFSCSVMHEALHNHYTQKSLSLSPGK

SEQ ID NO: 18 - protein, 213 aa, Artificial Sequence
  CHAIN (1)..(213): humanized Ab LC1
EIVLTQSPATLSLSPGERATLSCSASSSVIYMNWYQQKPGQAPRLLIYGISNLASGIPARFSGSGSGTDFTLTISSLEPEDFAVYYCQQRSSYPLTFGGGTKVEIKRTVAAPSVFIFPPSDEQLKSGTASVVCLLNNFYPREAKVQWKVDNALQSGNSQESVTEQDSKDSTYSLSSTLTLSKADYEKHKVYACEVTHQGLSSPVTKSFNRGEC

SEQ ID NO: 19 - protein, 213 aa, Artificial Sequence
  CHAIN (1)..(213): humanized Ab LC2
EIVLTQSPATLSLSPGERATLSCSASSSVIYMNWYQQKPGQSPKIWIYGISNLASGVPARFSGSGSGTDFTLTISSLEPEDFAVYYCQQRSSYPLTFGGGTKVEIKRTVAAPSVFIFPPSDEQLKSGTASVVCLLNNFYPREAKVQWKVDNALQSGNSQESVTEQDSKDSTYSLSSTLTLSKADYEKHKVYACEVTHQGLSSPVTKSFNRGEC

SEQ ID NO: 20 - protein, 213 aa, Artificial Sequence
  CHAIN (1)..(213): humanized Ab LC3
EILLTQSPATLSLSPGERATLTCSASSSVIYMNWYQQKPGSSPKIWIYGISNLASGVPARFSGSGSGTSFTLTISSLEPEDFAVYYCQQRSSYPLTFGGGTKVEIKRTVAAPSVFIFPPSDEQLKSGTASVVCLLNNFYPREAKVQWKVDNALQSGNSQESVTEQDSKDSTYSLSSTLTLSKADYEKHKVYACEVTHQGLSSPVTKSFNRGEC

SEQ ID NO: 21 - protein, 65 aa, Artificial Sequence
  PEPTIDE (1)..(65): hBCMA-His
MLQMAGQCSQNEYFDSLLHACIPCQLRCSSNTPPLTCQRYCNASVTNSVKGTNAHHHHHHHHHHH

SEQ ID NO: 22 - protein, 330 aa, Artificial Sequence [sequence omitted]

SEQ ID NO: 23 - protein, 107 aa, Artificial Sequence [sequence omitted]